European Patent Specification EP 3 885 367 B1, published June 10, 2026. Title: ANTI-HER2/PD1 BISPECIFIC ANTIBODY. Applicant: SUNSHINE GUOJIAN PHARMACEUTICAL (SHANGHAI) CO., LTD. The sequence listing filed with the application follows.

SEQUENCE LISTING (26 sequences)

SEQ ID NO: 1 - protein, 5 aa, Composite
SYDMS

SEQ ID NO: 2 - protein, 16 aa, Composite
TISGGGRYTYYPDTVK

SEQ ID NO: 3 - protein, 8 aa, Composite
PYGGYFDV

SEQ ID NO: 4 - protein, 11 aa, Composite
RASQSISNFLH

SEQ ID NO: 5 - protein, 7 aa, Composite
YASQSIS

SEQ ID NO: 6 - protein, 9 aa, Composite
QQSNSWPHT

SEQ ID NO: 7 - protein, 10 aa, Composite
GFNIKDTYIH

SEQ ID NO: 8 - protein, 17 aa, Composite
RIYPTNGYTRYADSVKG

SEQ ID NO: 9 - protein, 11 aa, Composite
WGGDGFYAMDY

SEQ ID NO: 10 - protein, 11 aa, Composite
RASQDVNTAVA

SEQ ID NO: 11 - protein, 8 aa, Composite
SASFLYSG

SEQ ID NO: 12 - protein, 9 aa, Composite
QQHYTTPPT

SEQ ID NO: 13 - protein, 117 aa, Composite
EVKLVESGGGLVQPGGSLRLSCAASGFAFSSYDMSWVRQAPGKRLEWVATISGGGRYTYYPDTVKGRFTISRDNAKNSHYLQMNSLRAEDTAVYFCASPYGGYFDVWGQGTLVTVSS

SEQ ID NO: 14 - protein, 107 aa, Composite
EIVLTQSPATLSLSPGERATLSCRASQSISNFLHWYQQKPGQAPRLLIKYASQSISGIPARFSGSGSGTDFTLTISSLEPEDFAVYFCQQSNSWPHTFGQGTKVEIK

SEQ ID NO: 15 - protein, 120 aa, Composite [sequence omitted]

SEQ ID NO: 16 - protein, 107 aa, Composite [sequence omitted]

SEQ ID NO: 17 - protein, 20 aa, Composite
GGGGSGGGGSGGGGSGGGGS

SEQ ID NO: 18 - protein, 15 aa, Composite
GGGGSGGGGSGGGGS

SEQ ID NO: 19 - protein, 244 aa, Composite
EIVLTQSPATLSLSPGERATLSCRASQSISNFLHWYQQKPGQAPRLLIKYASQSISGIPARFSGSGSGTDFTLTISSLEPEDFAVYFCQQSNSWPHTFGQGTKVEIKGGGGSGGGGSGGGGSGGGGSEVKLVESGGGLVQPGGSLRLSCAASGFAFSSYDMSWVRQAPGKRLEWVATISGGGRYTYYPDTVKGRFTISRDNAKNSHYLQMNSLRAEDTAVYFCASPYGGYFDVWGQGTLVTVSS

SEQ ID NO: 20 - protein, 709 aa, Composite
EVQLVESGGGLVQPGGSLRLSCAASGFNIKDTYIHWVRQAPGKGLEWVARIYPTNGYTRYADSVKGRFTISADTSKNTAYLQMNSLRAEDTAVYYCSRWGGDGFYAMDYWGQGTLVTVSSASTKGPSVFPLAPSSKSTSGGTAALGCLVKDYFPEPVTVSWNSGALTSGVHTFPAVLQSSGLYSLSSVVTVPSSSLGTQTYICNVNHKPSNTKVDKKVEPKSCDKTHTCPPCPAPELLGGPSVFLFPPKPKDTLMISRTPEVTCVVVDVSHEDPEVKFNWYVDGVEVHNAKTKPREEQYNSTYRVVSVLTVLHQDWLNGKEYKCKVSNKALPAPIEKTISKAKGQPREPQVYTLPPSREEMTKNQVSLTCLVKGFYPSDIAVEWESNGQPENNYKTTPPVLDSDGSFFLYSKLTVDKSRWQQGNVFSCSVMHEALHNHYTQKSLSLSPGKGGGGSGGGGSGGGGSEIVLTQSPATLSLSPGERATLSCRASQSISNFLHWYQQKPGQAPRLLIKYASQSISGIPARFSGSGSGTDFTLTISSLEPEDFAVYFCQQSNSWPHTFGQGTKVEIKGGGGSGGGGSGGGGSGGGGSEVKLVESGGGLVQPGGSLRLSCAASGFAFSSYDMSWVRQAPGKRLEWVATISGGGRYTYYPDTVKGRFTISRDNAKNSHYLQMNSLRAEDTAVYFCASPYGGYFDVWGQGTLVTVSS

SEQ ID NO: 21 - protein, 214 aa, Composite
DIQMTQSPSSLSASVGDRVTITCRASQDVNTAVAWYQQKPGKAPKLLIYSASFLYSGVPSRFSGSRSGTDFTLTISSLQPEDFATYYCQQHYTTPPTFGQGTKVEIKRTVAAPSVFIFPPSDEQLKSGTASVVCLLNNFYPREAKVQWKVDNALQSGNSQESVTEQDSKDSTYSLSSTLTLSKADYEKHKVYACEVTHQGLSSPVTKSFNRGEC

SEQ ID NO: 22 - DNA, 2127 bp, Composite
gaggtccaactggtggagtccggaggaggactggtgcaacccggcggatccctccggctgtcttgtgctgctagcggctttaacatcaaggatacctatatccattgggttaggcaagctcccggtaagggcttagaatgggtcgctaggatctaccccaccaatggctatactcgttacgccgacagcgtgaagggtcggttcaccatctccgctgacacctccaagaacacagcttacctccaaatgaactctttacgggccgaggacacagccgtgtactactgttcccggtggggaggcgacggcttctatgctatggattactggggccaaggtactttagtgacagtgtccagcgccagcacaaaaggaccttccgtcttccctctggctccctcctccaagagcaccagcggcggaacagctgctctcggctgtctggtgaaggactacttccccgaacccgttaccgtgtcttggaattccggcgctttaacctccggcgtgcacacctttcccgctgttttacagagcagcggcctctattctttaagctccgtggtcacagtgcctagcagctctttaggcacccagacctacatctgcaacgtgaaccataagcccagcaataccaaggtcgacaagaaggtggagcccaagagctgcgataagacccacacatgtcctccttgtcccgctcccgaactgctgggaggacccagcgtgtttttattcccccccaaacccaaagacaccctcatgatcagccggacccccgaggtcacatgcgtggtggtggacgtctcccacgaagaccccgaagtcaagttcaactggtacgtggacggagtcgaggtgcataacgccaagacaaaaccccgggaggagcaatacaactccacctatcgtgtggtgagcgtgctcaccgtgctgcatcaagattggctgaatggcaaggagtacaagtgcaaggtcagcaacaaggctctgcccgctcctatcgagaagacaatcagcaaagccaaaggccaaccccgggagccccaagtgtatactttacccccctcccgggaagagatgaccaagaaccaagtttctttaacatgtttagtgaaaggcttttacccctccgacatcgccgtcgagtgggagtccaatggccagcccgaaaataactacaagacaaccccccccgtgctcgattccgatggatccttctttttatacagcaagctcacagtggataagtcccggtggcagcaaggaaacgtgttttcttgttccgtcatgcacgaggccctccataaccactacacccagaaatccctctctctcagccccggtaaaggcggaggaggatccggcggcggcggaagcggaggaggcggctccgagatcgtgctgacccagtcccccgctacactgtccctctctcccggtgaacgggctactttaagctgtcgtgccagccaaagcatcagcaactttttacactggtaccaacagaaacccggccaagctccccggctgctgatcaagtacgcttcccagagcatcagcggcattcccgctaggttctccggcagcggcagcggaaccgatttcactttaaccatcagctctttagagcccgaggacttcgccgtctacttctgccaacagagcaatagctggcctcacacattcggccaaggtacaaaggtcgagatcaaaggtggaggtggcagcggtggcggcggcagcggtggtggtggaagcggaggcggaggctccgaggtgaagctcgtggaatctggcggaggtttagtgcagcccggtggctctttaaggctgagctgtgctgccagcggctttgcctttagctcctacgacatgagctgggtgcgtcaagctcccggaaagaggctggagtgggtggccacaatctccggcggtggtcgttatacctattaccccgacaccgtcaaaggccggtttaccatcagccgggacaacgctaagaacagccattacctccagatgaattctttacgggctgaggacaccgctgtgtatttctgtgctagcccctacggcggctactttgatgtctggggacaaggtaccctcgtgaccgtgagctcc

SEQ ID NO: 23 - DNA, 642 bp, Composite
gacatccagatgacacagagcccctcctctttatccgcttccgtgggagatcgtgtcaccatcacttgtcgtgcctcccaagatgtgaacaccgctgtggcttggtaccagcagaagcccggtaaggctcccaagctgctgatctactccgccagctttttatactccggcgtgccctctcgtttctccggatctcgttccggcaccgacttcactttaaccatcagctctttacagcccgaggacttcgccacctactactgccagcagcactacaccaccccccctaccttcggacaaggtaccaaggtggagatcaagaggaccgtggccgccccctccgtcttcatctttcccccttccgacgagcagctgaagtccggcacagcctccgtggtgtgtttactgaataacttctacccccgggaggccaaggtgcagtggaaggtggataacgctttacagtccggcaacagccaagaaagcgtgaccgaacaagatagcaaggactccacctactctttatcctccactttaactttaagcaaggccgactacgagaagcataaggtgtacgcttgtgaggtgacccatcaaggtttaagcagccccgtgaccaagtccttcaaccggggcgaatgc

SEQ ID NO: 24 - protein, 244 aa, Composite
EVKLVESGGGLVQPGGSLRLSCAASGFAFSSYDMSWVRQAPGKRLEWVATISGGGRYTYYPDTVKGRFTISRDNAKNSHYLQMNSLRAEDTAVYFCASPYGGYFDVWGQGTLVTVSSGGGGSGGGGSGGGGSGGGGSEIVLTQSPATLSLSPGERATLSCRASQSISNFLHWYQQKPGQAPRLLIKYASQSISGIPARFSGSGSGTDFTLTISSLEPEDFAVYFCQQSNSWPHTFGQGTKVEIK

SEQ ID NO: 25 - protein, 709 aa, Composite
EVKLVESGGGLVQPGGSLRLSCAASGFAFSSYDMSWVRQAPGKRLEWVATISGGGRYTYYPDTVKGRFTISRDNAKNSHYLQMNSLRAEDTAVYFCASPYGGYFDVWGQGTLVTVSSGGGGSGGGGSGGGGSGGGGSEIVLTQSPATLSLSPGERATLSCRASQSISNFLHWYQQKPGQAPRLLIKYASQSISGIPARFSGSGSGTDFTLTISSLEPEDFAVYFCQQSNSWPHTFGQGTKVEIKGGGGSGGGGSGGGGSEVQLVESGGGLVQPGGSLRLSCAASGFNIKDTYIHWVRQAPGKGLEWVARIYPTNGYTRYADSVKGRFTISADTSKNTAYLQMNSLRAEDTAVYYCSRWGGDGFYAMDYWGQGTLVTVSSASTKGPSVFPLAPSSKSTSGGTAALGCLVKDYFPEPVTVSWNSGALTSGVHTFPAVLQSSGLYSLSSVVTVPSSSLGTQTYICNVNHKPSNTKVDKKVEPKSCDKTHTCPPCPAPELLGGPSVFLFPPKPKDTLMISRTPEVTCVVVDVSHEDPEVKFNWYVDGVEVHNAKTKPREEQYNSTYRVVSVLTVLHQDWLNGKEYKCKVSNKALPAPIEKTISKAKGQPREPQVYTLPPSREEMTKNQVSLTCLVKGFYPSDIAVEWESNGQPENNYKTTPPVLDSDGSFFLYSKLTVDKSRWQQGNVFSCSVMHEALHNHYTQKSLSLSPGK

SEQ ID NO: 26 - DNA, 2127 bp, Composite
gaggtgaagctggtggagtccggcggcggcctggtgcagcctggcggctccctgaggctgtcctgcgccgcctccggcttcgccttctcctcctacgacatgtcctgggtgaggcaggcccctggcaagaggctggagtgggtggccaccatctccggcggcggcaggtacacctactaccctgacaccgtgaagggcaggttcaccatctccagggacaacgccaagaactcccactacctgcagatgaactccctgagggccgaggacaccgccgtgtacttctgcgcctccccttacggcggctacttcgacgtgtggggccagggcaccctggtgaccgtgtcctccggcggcggcggctccggcggcggcggctccggcggcggcggctccggcggcggcggctccgagatcgtgctgacccagtcccctgccaccctgtccctgtcccctggcgagagggccaccctgtcctgcagggcctcccagtccatctccaacttcctgcactggtaccagcagaagcctggccaggcccctaggctgctgatcaagtacgcctcccagtccatctccggcatccctgccaggttctccggctccggctccggcaccgacttcaccctgaccatctcctccctggagcctgaggacttcgccgtgtacttctgccagcagtccaactcctggcctcacaccttcggccagggcaccaaggtggagatcaagggcggcggcggctccggcggcggcggctccggcggcggcggctccgaggtccaactggtggagtccggaggaggactggtgcaacccggcggatccctccggctgtcttgtgctgctagcggctttaacatcaaggatacctatatccattgggttaggcaagctcccggtaagggcttagaatgggtcgctaggatctaccccaccaatggctatactcgttacgccgacagcgtgaagggtcggttcaccatctccgctgacacctccaagaacacagcttacctccaaatgaactctttacgggccgaggacacagccgtgtactactgttcccggtggggaggcgacggcttctatgctatggattactggggccaaggtactttagtgacagtgtccagcgccagcacaaaaggaccttccgtcttccctctggctccctcctccaagagcaccagcggcggaacagctgctctcggctgtctggtgaaggactacttccccgaacccgttaccgtgtcttggaattccggcgctttaacctccggcgtgcacacctttcccgctgttttacagagcagcggcctctattctttaagctccgtggtcacagtgccttcctcctccctgggcacccagacctacatctgcaacgtgaaccacaagccttccaacaccaaggtggacaagaaggtggagcctaagtcctgcgacaagacccacacctgccctccttgccctgcccctgagctgctgggcggcccttccgtgttcctgttccctcctaagcctaaggacaccctgatgatctccaggacccctgaggtgacctgcgtggtggtggacgtgtcccacgaggaccctgaggtgaagttcaactggtacgtggacggcgtggaggtgcacaacgccaagaccaagcctagggaggagcagtacaactccacctacagggtggtgtccgtgctgaccgtgctgcaccaggactggctgaacggcaaggagtacaagtgcaaggtgtccaacaaggccctgcctgcccctatcgagaagaccatctccaaggccaagggccagcctagggagcctcaggtgtacaccctgcctccttccagggaggagatgaccaagaaccaggtgtccctgacctgcctggtgaagggcttctacccttccgacatcgccgtggagtgggagtccaacggccagcctgagaacaactacaagaccacccctcctgtgctggactccgacggctccttcttcctgtactccaagctgaccgtggacaagtccaggtggcagcagggcaacgtgttctcctgctccgtgatgcacgaggccctgcacaaccactacacccagaagtccctgtccctgtcccctggcaag